European Patent Specification EP 3 344 284 B1, published May 20, 2026. Title: IMMUNE CELL COMPOSITIONS AND METHODS OF USE. Applicant: MEMORIAL SLOAN KETTERING CANCER CENTER. The sequence listing filed with the application follows.

SEQUENCE LISTING (48 sequences)

SEQ ID NO: 1 - protein, 164 aa, Homo sapiens
MKWKALFTAAILQAQLPITEAQSFGLLDPKLCYLLDGILFIYGVILTALFLRVKFSRSADAPAYQQGQNQLYNELNLGRREEYDVLDKRRGRDPEMGGKPQRRKNPQEGLYNELQKDKMAEAYSEIGMKGERRRGKGHDGLYQGLSTATKDTYDALHMQALPPR

SEQ ID NO: 2 - DNA, 339 bp, Homo sapiens
agagtgaagttcagcaggagcgcagacgcccccgcgtaccagcagggccagaaccagctctataacgagctcaatctaggacgaagagaggagtacgatgttttggacaagagacgtggccgggaccctgagatggggggaaagccgagaaggaagaaccctcaggaaggcctgtacaatgaactgcagaaagataagatggcggaggcctacagtgagattgggatgaaaggcgagcgccggaggggcaaggggcacgatggcctttaccagggtctcagtacagccaccaaggacacctacgacgcccttcacatgcaggccctgccccctcgctaa

SEQ ID NO: 3 - protein, 220 aa, Homo sapiens
MLRLLLALNLFPSIQVTGNKILVKQSPMLVAYDNAVNLSCKYSYNLFSREFRASLHKGLDSAVEVCVVYGNYSQQLQVYSKTGFNCDGKLGNESVTFYLQNLYVNQTDIYFCKIEVMYPPPYLDNEKSNGTIIHVKGKHLCPSPLFPGPSKPFWVLVVVGGVLACYSLLVTVAFIIFWVRSKRSRLLHSDYMNMTPRRPGPTRKHYQPYAPPRDFAAYRS

SEQ ID NO: 4 - DNA, 321 bp, Homo sapiens
attgaagttatgtatcctcctccttacctagacaatgagaagagcaatggaaccattatccatgtgaaagggaaacacctttgtccaagtcccctatttcccggaccttctaagcccttttgggtgctggtggtggttggtggagtcctggcttgctatagcttgctagtaacagtggcctttattattttctgggtgaggagtaagaggagcaggctcctgcacagtgactacatgaacatgactccccgccgccccgggcccacccgcaagcattaccagccctatgccccaccacgcgacttcgcagcctatcgctcc

SEQ ID NO: 5 - protein, 255 aa, Homo sapiens
MGNSCYNIVATLLLVLNFERTRSLQDPCSNCPAGTFCDNNRNQICSPCPPNSFSSAGGQRTCDICRQCKGVFRTRKECSSTSNAECDCTPGFHCLGAGCSMCEQDCKQGQELTKKGCKDCCFGTFNDQKRGICRPWTNCSLDGKSVLVNGTKERDVVCGPSPADLSPGASSVTPPAPAREPGHSPQIISFFLALTSTALLFLLFFLTLRFSVVKRGRKKLLYIFKQPFMRPVQTTQEEDGCSCRFPEEEEGGCEL

SEQ ID NO: 6 - protein, 277 aa, Homo sapiens
MCVGARRLGRGPCAALLLLGLGLSTVTGLHCVGDTYPSNDRCCHECRPGNGMVSRCSRSQNTVCRPCGPGFYNDVVSSKPCKPCTWCNLRSGSERKQLCTATQDTVCRCRAGTQPLDSYKPGVDCAPCPPGHFSPGDNQACKPWTNCTLAGKHTLQPASNSSDAICEDRDPPATQPQETQGPPARPITVQPTEAWPRTSQGPSTRPVEVPGGRAVAAILGLGLVLGLLGPLAILLALYLLRRDQRLPPDAHKPPGGGSFRTPIQEEQADAHSTLAKI

SEQ ID NO: 7 - protein, 199 aa, Homo sapiens
MKSGLWYFFLFCLRIKVLTGEINGSANYEMFIFHNGGVQILCKYPDIVQQFKMQLLKGGQILCDLTKTKGSGNTVSIKSLKFCHSQLSNNSVSFFLYNLDHSHANYYFCNLSIFDPPPFKVTLTGGYLHIYESQLCCQLKFWLPIGCAAFVVVCILGCILICWLTKKKYSSSVHDPNGEYMFMRAVNTAKKSRLTDVTL

SEQ ID NO: 8 - protein, 93 aa, Homo sapiens
MIHLGHILFLLLLPVAAAQTTPGERSSLPAFYPGTSGSCSGCGSLSLPLLAGLVAADAVASLLIVGAVFLCARPRRSPAQEDGKVYINMPGRG

SEQ ID NO: 9 - protein, 21 aa, Homo sapiens
MALPVTALLLPLALLLHAARP

SEQ ID NO: 10 - protein, 15 aa, Artificial Sequence
  Description of Artificial Sequence: Synthetic peptide
GGGGSGGGGSGGGGS

SEQ ID NO: 11 - protein, 235 aa, Homo sapiens
MALPVTALLLPLALLLHAARPSQFRVSPLDRTWNLGETVELKCQVLLSNPTSGCSWLFQPRGAAASPTFLLYLSQNKPKAAEGLDTQRFSGKRLGDTFVLTLSDFRRENEGYYFCSALSNSIMYFSHFVPVFLPAKPTTTPAPRPPTPAPTIASQPLSLRPEACRPAAGGAVHTRGLDFACDIYIWAPLAGTCGVLLLSLVITLYCNHRNRRRVCKCPRPVVKSGDKPSLSARYV

SEQ ID NO: 12 - protein, 458 aa, Homo sapiens
MNRGVPFRHLLLVLQLALLPAATQGKKVVLGKKGDTVELTCTASQKKSIQFHWKNSNQIKILGNQGSFLTKGPSKLNDRADSRRSLWDQGNFPLIIKNLKIEDSDTYICEVEDQKEEVQLLVFGLTANSDTHLLQGQSLTLTLESPPGSSPSVQCRSPRGKNIQGGKTLSVSQLELQDSGTWTCTVLQNQKKVEFKIDIVVLAFQKASSIVYKKEGEQVEFSFPLAFTVEKLTGSGELWWQAERASSSKSWITFDLKNKEVSVKRVTQDPKLQMGKKLPLHLTLPQALPQYAGSGNLTLALEAKTGKLHQEVNLVVMRATQLQKNLTCEVWGPTSPKLMLSLKLENKEAKVSKREKAVWVLNPEAGMWQCLLSDSGQVLLESNIKVLPTWSTPVQPMALIVLGGVAGLLLFIGLGIFFCVRCRHRRRQAERMSQIKRLLSEKKTCQCPHRFQKTCSPI

SEQ ID NO: 13 - protein, 622 aa, Homo sapiens [sequence omitted]

SEQ ID NO: 14 - protein, 230 aa, Artificial Sequence
  Description of Artificial Sequence: Synthetic polypeptide
QVQLQESGPGLVKPSETLSLTCTVSGGSVSSGSYYWSWIRQPPGKGLEWIGYIYYSGSTNYNPSLKSRVTISVDTSKNQFSLKLSSVTAADTAVYYCAREGKNGAFDIWGQGTMVTVSSASTKGPSVFPLAPSSKSTSGGTAALGCLVKDYFPEPVTVSWNSGALTSGVHTFPAVLQSSGLYSLSSVVTVPSSSLGTQTYICNVNHKPSNTKVDKKVEPKSCDKTSGQAG

SEQ ID NO: 15 - DNA, 693 bp, Artificial Sequence
  Description of Artificial Sequence: Synthetic polynucleotide
caggtgcagctgcaggagtccggcccaggactggtgaagccttcggagaccctgtccctcacctgcactgtctctggtggctccgtcagcagtggtagttactactggagctggatccggcagcccccagggaagggactggagtggattgggtatatctattacagtgggagcaccaactacaacccctccctcaagagtcgagtcaccatatcagtagacacgtccaagaaccagttctccctgaagctgagctctgtgaccgctgcggacacggccgtgtattactgtgcgagagaggggaagaatggggcttttgatatctggggccaagggacaatggtcaccgtctcttcagcctccaccaagggcccatcggtcttccccctggcaccctcctccaagagcacctctgggggcacagcggccctgggctgcctggtcaaggactacttccccgaaccggtgacggtgtcgtggaactcaggcgccctgaccagcggcgtgcacaccttcccggctgtcctacagtcctcaggactctactccctcagcagcgtggtgaccgtgccctccagcagcttgggcacccagacctacatctgcaacgtgaatcacaagcccagcaacaccaaggtggacaagaaagttgagcccaaatcttgtgacaaaactagtggccaggccggccac

SEQ ID NO: 16 - protein, 214 aa, Artificial Sequence
  Description of Artificial Sequence: Synthetic polypeptide
DIQMTQSPSSLSASVGDRVTITCRASQSISSYLNWYQQKPGKAPKLLIYAASSLQSGVPSGFSGSGSGTDFTLTISSLQPEDFATYYCQQSYSTPLTFGGGTKVEIKRTVAAPSVFIFPPSDEQLKSGTASVVCLLNNFYPREAKVQWKVDNALQSGNSQESVTEQDSKDSTYSLSSTLTLSKADYEKHKVYACEVTHQGLSSPVTKSFNRGEC

SEQ ID NO: 17 - DNA, 640 bp, Artificial Sequence
  Description of Artificial Sequence: Synthetic polynucleotide
gacatccagatgacccagtctccatcctccctgtctgcatctgtaggagacagagtcaccatcacttgccgggcaagtcagagcattagcagctatttaaattggtatcagcagaaaccagggaaagcccctaagctcctgatctatgctgcatccagtttgcaaagtggggtcccatcagggttcagtggcagtggatctgggacagatttcactctcaccatcagcagtctgcaacctgaagattttgcaacttactactgtcaacagagttacagtaccccgctcactttcggcggagggaccaaggtggagatcaaacgaactgtggctgcaccatctgtcttcatcttcccgccatctgatgagcagttgaaatctggaactgcctctgttgtgtgcctgctgaataacttctatcccagagaggccaaagtacagtggaaggtggataacgccctccaatcgggtaactcccaggagagtgtcacagagcaggacagcaaggacagcacctactgcctcagcagcaccctgacgctgagcaaagcagactacgagaaacacaaactctacgcctgcgaagtcacccatcagggcctgagctcgcccgtcacaaagagcttcaacaggggagagt

SEQ ID NO: 18 - protein, 214 aa, Artificial Sequence
  Description of Artificial Sequence: Synthetic polypeptide
RHQMTQSPSSLSASVGDRVTITCRASQSISSYLNWYQQKPGKAPKLLIYAASSLQSGVPSGFSGSGSGTDFTLTISSLQPEDFATYYCQQSYSTPLTFGGGTKVEIKRTVAAPSVFIFPPSDEQLKSGTASVVCLLNNFYPREAKVQWKVDNALQSGNSQESVTEQDSKDSTYSLSSTLTLSKADYEKHKVYACEVTHQGLSSPVTKSFNRGEC

SEQ ID NO: 19 - protein, 120 aa, Artificial Sequence
  Description of Artificial Sequence: Synthetic polypeptide
QVQLQESGPGLVKPSETLSLTCTVSGGSVSSGSYYWSWIRQPPGKGLEWIGYIYYSGSTNYNPSLKSRVTISVDTSKNQFSLKLSSVTAADTAVYYCAREGKNGAFDIWGQGTMVTVSSS

SEQ ID NO: 20 - protein, 262 aa, Homo sapiens
QVQLQESGPGLVKPSETLSLTCTVSGGSVSSGSYYWSWIRQPPGKGLEWIGYIYYSGSTNYNPSLKSRVTISVDTSKNQFSLKLSSVTAADTAVYYCAREGKNGAFDIWGQGTMVTVSSSGGGGSGGGGSGGGGSRHQMTQSPSSLSASVGDRVTITCRASQSISSYLNWYQQKPGKAPKLLIYAASSLQSGVPSRFSGSGSGTDFTLTISSLQPEDFATYYCQQSYSTPLTFGGGTKVEIKGQAGHHHHHHGDYKDDDDKG

SEQ ID NO: 21 - DNA, 801 bp, Homo sapiens
atggccttaccagtgaccgccttgctcctgccgctggccttgctgctccacgccgccaggccgcaggtgcagctgcaggagtccggcccaggactggtgaagccttcggagaccctgtccctcacctgcactgtctctggtggctccgtcagcagtggtagttactactggagctggatccggcagcccccagggaagggactggagtggattgggtatatctattacagtgggagcaccaactacaacccctccctcaagagtcgagtcaccatatcagtagacacgtccaagaaccagttctccctgaagctgagctctgtgaccgctgcggacacggccgtgtattactgtgcgagagaggggaagaatggggcttttgatatctggggccaagggacaatggtcaccgtctcttcaggtggaggcggttcaggcggaggtggctctggcggtggcggatcacgacatcagatgacccagtctccatcctccctgtctgcatctgtaggagacagagtcaccatcacttgccgggcaagtcagagcattagcagctatttaaattggtatcagcagaaaccagggaaagcccctaagctcctgatctatgctgcatccagtttgcaaagtggggtcccatcaaggttcagtggcagtggatctgggacagatttcactctcaccatcagcagtctgcaacctgaagattttgcaacttactactgtcaacagagttacagtaccccgctcactttcggcggagggaccaaggtggagatcaaacggactgcggccgca

SEQ ID NO: 22 - DNA, 801 bp, Artificial Sequence
  Description of Artificial Sequence: Synthetic polynucleotide
atggcgctgccggtgaccgcgctgctgctgccgctggcgctgctgctgcatgcggcgcgcccgcaggtgcagctgcaggaaagcggcccgggcctggtgaaaccgagcgaaaccctgagcctgacctgcaccgtgagcggcggcagcgtgagcagcggcagctattattggagctggattcgccagccgccgggcaaaggcctggaatggattggctatatttattatagcggcagcaccaactataacccgagcctgaaaagccgcgtgaccattagcgtggataccagcaaaaaccagtttagcctgaaactgagcagcgtgaccgcggcggataccgcggtgtattattgcgcgcgcgaaggcaaaaacggcgcgtttgatatttggggccagggcaccatggtgaccgtgagcagcggcggcggcggcagcggcggcggcggcagcggcggcggcggcagccgccatcagatgacccagagcccgagcagcctgagcgcgagcgtgggcgatcgcgtgaccattacctgccgcgcgagccagagcattagcagctatctgaactggtatcagcagaaaccgggcaaagcgccgaaactgctgatttatgcggcgagcagcctgcagagcggcgtgccgagccgctttagcggcagcggcagcggcaccgattttaccctgaccattagcagcctgcagccggaagattttgcgacctattattgccagcagagctatagcaccccgctgacctttggcggcggcaccaaagtggaaattaaacgcaccgcggcggcg

SEQ ID NO: 23 - DNA, 801 bp, Artificial Sequence
  Description of Artificial Sequence: Synthetic polynucleotide
atggccctcccggtaacggctctgctgcttccactcgcactgctcttgcatgctgccagaccacaggtccagctgcaggagagtgggcctggactggttaagccgagtgagacactttccttgacgtgcactgtgagcgggggaagtgtgtcctcaggtagttattactggtcctggattcgccagccaccaggaaagggactggagtggataggttatatctattattctggcagcactaattacaatccttctctcaaaagtagggtgacaatttcagtggatacttccaaaaatcagtttagtctgaagctcagctctgtgacagctgctgatactgcagtttactactgcgccagggaggggaagaatggcgccttcgatatttggggacagggcactatggtgactgtatcaagcggaggcggtggcagcggcgggggagggagtggaggcggcgggtctcgacatcagatgacacagagcccatcatcacttagcgccagcgttggcgaccgggttacgataacatgcagggcttcccaatctatcagttcttatctgaactggtatcagcagaaaccaggtaaggcccccaagctgctcatctacgcagcctcatccctgcagagcggcgtccctagtcgattttccggtagtgggtcagggacagattttaccctgactatcagttcactgcagcccgaggacttcgcgacatactattgccaacagtcctatagtacacccttgacatttggcggcgggactaaagtagaaattaaacgcaccgcggccgca

SEQ ID NO: 24 - protein, 10 aa, Artificial Sequence
  Description of Artificial Sequence: Synthetic peptide
GGSVSSGSYY

SEQ ID NO: 25 - protein, 7 aa, Artificial Sequence
  Description of Artificial Sequence: Synthetic peptide
IYYSGST

SEQ ID NO: 26 - protein, 12 aa, Artificial Sequence
  Description of Artificial Sequence: Synthetic peptide
AREGKNGAFDIW

SEQ ID NO: 27 - protein, 6 aa, Artificial Sequence
  Description of Artificial Sequence: Synthetic peptide
QSISSY

SEQ ID NO: 28 - protein, 4 aa, Artificial Sequence
  Description of Artificial Sequence: Synthetic peptide
AASS

SEQ ID NO: 29 - protein, 10 aa, Artificial Sequence
  Description of Artificial Sequence: Synthetic peptide
QQSYSTPLTF

SEQ ID NO: 30 - protein, 21 aa, Homo sapiens
MALPVTALLLPLALLLHAARP

SEQ ID NO: 31 - protein, 21 aa, Homo sapiens
MALPVTALLLPLALLLHAARP

SEQ ID NO: 32 - protein, 21 aa, Homo sapiens
MALPVTALLLPLALLLHAARP

SEQ ID NO: 33 - protein, 288 aa, Homo sapiens
MQIPQAPWPVVWAVLQLGWRPGWFLDSPDRPWNPPTFSPALLVVTEGDNATFTCSFSNTSESFVLNWYRMSPSNQTDKLAAFPEDRSQPGQDCRFRVTQLPNGRDFHMSVVRARRNDSGTYLCGAISLAPKAQIKESLRAELRVTERRAEVPTAHPSPSPRPAGQFQTLVVGVVGGLLGSLVLLVWVLAVICSRAARGTIGARRTGQPLKEDPSAVPVFSVDYGELDFQWREKTPEPPVPCVPEQTEYATIVFPSGMGTSSPARRGSADGPRSAQPLRPEDGHCSWPL

SEQ ID NO: 34 - protein, 223 aa, Homo sapiens
MACLGFQRHKAQLNLATRTWPCTLLFFLLFIPVFCKAMHVAQPAVVLASSRGIASFVCEYASPGKATEVRVTVLRQADSQVTEVCAATYMMGNELTFLDDSICTGTSSGNQVNLTIQGLRAMDTGLYICKVELMYPPPYYLGIGNGTQIYVIDPEPCPDSDFLLWILAAVSSGLFFYSFLLTAVSLSKMLKKRSPLTTGVYVKMPPTEPECEKQFQPYFIPIN

SEQ ID NO: 35 - protein, 289 aa, Homo sapiens
MKTLPAMLGTGKLFWVFFLIPYLDIWNIHGKESCDVQLYIKRQSEHSILAGDPFELECPVKYCANRPHVTWCKLNGTTCVKLEDRQTSWKEEKNISFFILHFEPVLPNDNGSYRCSANFQSNLIESHSTTLYVTDVKSASERPSKDEMASRPWLLYSLLPLGGLPLLITTCFCLFCCLRRHQGKQNELSDTAGREINLVDAHLKSEQTEASTRQNSQVLLSETGIYDNDPDLCFRMQEGSEVYSNPCLEENKPGIVYASLNHSVIGPNSRLARNVKEAPTEYASICVRS

SEQ ID NO: 36 - protein, 301 aa, Homo sapiens
MFSHLPFDCVLLLLLLLLTRSSEVEYRAEVGQNAYLPCFYTPAAPGNLVPVCWGKGACPVFECGNVVLRTDERDVNYWTSRYWLNGDFRKGDVSLTIENVTLADSGIYCCRIQIPGIMNDEKFNLKLVIKPAKVTPAPTRQRDFTAAFPRMLTTRGHGPAETQTLGSLPDINLTQISTLANELRDSRLANDLRDSGATIRIGIYIGAGICAGLALALIFGALIFKWYSHSKEKIQNLSLISLANLPPSGLANAVAEGIRSEENIYTIEENVYEVEEPNEYYCYVSSRQQPSQPLGCRFAMP

SEQ ID NO: 37 - protein, 525 aa, Homo sapiens
MWEAQFLGLLFLQPLWVAPVKPLQPGAEVPVVWAQEGAPAQLPCSPTIPLQDLSLLRRAGVTWQHQPDSGPPAAAPGHPLAPGPHPAAPSSWGPRPRRYTVLSVGPGGLRSGRLPLQPRVQLDERGRQRGDFSLWLRPARRADAGEYRAAVHLRDRALSCRLRLRLGQASMTASPPGSLRASDWVILNCSFSRPDRPASVHWFRNRGQGRVPVRESPHHHLAESFLFLPQVSPMDSGPWGCILTYRDGFNVSIMYNLTVLGLEPPTPLTVYAGAGSRVGLPCRLPAGVGTRSFLTAKWTPPGGGPDLLVTGDNGDFTLRLEDVSQAQAGTYTCHIHLQEQQLNATVTLAIITVTPKSFGSPGSLGKLLCEVTPVSGQERFVWSSLDTPSQRSFSGPWLEAQEAQLLSQPWQCQLYQGERLLGAAVYFTELSSPGAQRSGRAPGALPAGHLLLFLILGVLSLLLLVTGAFGFHLWRRQWRPRRFSALEQGIHPPQAQSKIEELEQEPEPEPEPEPEPEPEPEPEQL

SEQ ID NO: 38 - protein, 244 aa, Homo sapiens
MRWCLLLIWAQGLRQAPLASGMMTGTIETTGNISAEKGGSIILQCHLSSTTAQVTQVNWEQQDQLLAICNADLGWHISPSFKDRVAPGPGLGLTLQSLTVNDTGEYFCIYHTYPDGTYTGRIFLEVLESSVAEHGARFQIPLLGAMAATLVVICTAVIVVVALTRKKKALRIHSVEGDLRRKSAGQEEWSPSAPSPPGSCVQAEAAPAGLCGEQRGEDCAELHDYFNVLSYRSLGNCSFFTETG

SEQ ID NO: 39 - protein, 287 aa, Homo sapiens
MSPHPTALLGLVLCLAQTIHTQEEDLPRPSISAEPGTVIPLGSHVTFVCRGPVGVQTFRLERDSRSTYNDTEDVSQASPSESEARFRIDSVREGNAGLYRCIYYKPPKWSEQSDYLELLVKESSGGPDSPDTEPGSSAGPTQRPSDNSHNEHAPASQGLKAEHLYILIGVSVVFLFCLLLLVLFCLHRQNQIKQGPPRSKDEEQKPQQRPDLAVDVLERTADKATVNGLPEKDRETDTSALAAGSSQEVTYAQLDHWALTQRTARAVSPQSTKPMAESITYAAVARH

SEQ ID NO: 40 - protein, 370 aa, Homo sapiens
MLGQVVTLILLLLLKVYQGKGCQGSADHVVSISGVPLQLQPNSIQTKVDSIAWKKLLPSQNGFHHILKWENGSLPSNTSNDRFSFIVKNLSLLIKAAQQQDSGLYCLEVTSISGKVQTATFQVFVFESLLPDKVEKPRLQGQGKILDRGRCQVALSCLVSRDGNVSYAWYRGSKLIQTAGNLTYLDEEVDINGTHTYTCNVSNPVSWESHTLNLTQDCQNAHQEFRFWPFLVIIVILSALFLGTLACFCVWRRKRKEKQSETSPKEFLTIYEDVKDLKTRRNHEQEQTFPGGGSTIYSMIQSQSSAPTSQEPAYTLYSLIQPSRKSGSRKRNHSPSFNSTIYEVIGKSQPKAQNPARLSRKELENFDVYS

SEQ ID NO: 41 - protein, 181 aa, Homo sapiens
MLLEPGRGCCALAILLAIVDIQSGGCINITSSASQEGTRLNLICTVWHKKEEAEGFVVFLCKDRSGDCSPETSLKQLRLKRDPGIDGVGEISSQLMFTISQVTPLHSGTYQCCARSQKSGIRLQGHFFSILFTETGNYTVTGLKQRQHLEFSHNEGTLSSGFLQEKVWVMLVTSLVALQAL

SEQ ID NO: 42 - protein, 592 aa, Homo sapiens
MGRGLLRGLWPLHIVLWTRIASTIPPHVQKSDVEMEAQKDEIICPSCNRTAHPLRHINNDMIVTDNNGAVKFPQLCKFCDVRFSTCDNQKSCMSNCSITSICEKPQEVCVAVWRKNDENITLETVCHDPKLPYHDFILEDAASPKCIMKEKKKPGETFFMCSCSSDECNDNIIFSEEYNTSNPDLLLVIFQVTGISLLPPLGVAISVIIIFYCYRVNRQQKLSSTWETGKTRKLMEFSEHCAIILEDDRSDISSTCANNINHNTELLPIELDTLVGKGRFAEVYKAKLKQNTSEQFETVAVKIFPYEEYASWKTEKDIFSDINLKHENILQFLTAEERKTELGKQYWLITAFHAKGNLQEYLTRHVISWEDLRKLGSSLARGIAHLHSDHTPCGRPKMPIVHRDLKSSNILVKNDLTCCLCDFGLSLRLDPTLSVDDLANSGQVGTARYMAPEVLESRMNLENVESFKQTDVYSMALVLWEMTSRCNAVGEVKDYEPPFGSKVREHPCVESMKDNVLRDRGRPEIPSFWLNHQGIQMVCETLTECWDHDPEARLTAQCVAERFSELEHLDRLSGRSCSEEKIPEDGSLNTTK

SEQ ID NO: 43 - protein, 244 aa, Artificial Sequence
  Description of Artificial Sequence: Synthetic polypeptide
MQIPQAPWPVVWAVLQLGWRPGWFLDSPDRPWNPPTFSPALLVVTEGDNATFTCSFSNTSESFVLNWYRMSPSNQTDKLAAFPEDRSQPGQDCRFRVTQLPNGRDFHMSVVRARRNDSGTYLCGAISLAPKAQIKESLRAELRVTERRAEVPTAHPSPSPRPAGQAAAPTTTPAPRPPTPAPTIASQPLSLRPEACRPAAGGAVHTRGLDFACDIYIWAPLAGTCGVLLLSLVITLYCNHRRIQ

SEQ ID NO: 44 - protein, 23 aa, Artificial Sequence
  Description of Artificial Sequence: Synthetic peptide
GSGATNFSLLKQAGDVEENPGPM

SEQ ID NO: 45 - protein, 236 aa, Artificial Sequence
  Description of Artificial Sequence: Synthetic polypeptide
MVSKGEEDNMAIIKEFMRFKVHMEGSVNGHEFEIEGEGEGRPYEGTQTAKLKVTKGGPLPFAWDILSPQFMYGSKAYVKHPADIPDYLKLSFPEGFKWERVMNFEDGGVVTVTQDSSLQDGEFIYKVKLRGTNFPSDGPVMQKKTMGWEASSERMYPEDGALKGEIKQRLKLKDGGHYDAEVKTTYKAKKPVQLPGAYNVNIKLDITSHNEDYTIVEQYERAEGRHSTGGMDELYK

SEQ ID NO: 46 - protein, 502 aa, Artificial Sequence
  Description of Artificial Sequence: Synthetic polypeptide
MQIPQAPWPVVWAVLQLGWRPGWFLDSPDRPWNPPTFSPALLVVTEGDNATFTCSFSNTSESFVLNWYRMSPSNQTDKLAAFPEDRSQPGQDCRFRVTQLPNGRDFHMSVVRARRNDSGTYLCGAISLAPKAQIKESLRAELRVTERRAEVPTAHPSPSPRPAGQAAAPTTTPAPRPPTPAPTIASQPLSLRPEACRPAAGGAVHTRGLDFACDIYIWAPLAGTCGVLLLSLVITLYCNHRRIQGSGATNFSLLKQAGDVEENPGPMVSKGEEDNMAIIKEFMRFKVHMEGSVNGHEFEIEGEGEGRPYEGTQTAKLKVTKGGPLPFAWDILSPQFMYGSKAYVKHPADIPDYLKLSFPEGFKWERVMNFEDGGVVTVTQDSSLQDGEFIYKVKLRGTNFPSDGPVMQKKTMGWEASSERMYPEDGALKGEIKQRLKLKDGGHYDAEVKTTYKAKKPVQLPGAYNVNIKLDITSHNEDYTIVEQYERAEGRHSTGGMDELYK

SEQ ID NO: 47 - DNA, 1726 bp, Artificial Sequence
  Description of Artificial Sequence: Synthetic polynucleotide
accggtggtacctcacccttaccgagtcggcgacacagtgtgggtccgccgacaccagactaagaacctagaacctcgctggaaaggaccttacacagtcctgctgaccacccccaccgccctcaaagtagacggcatcgcagcttggatacacgccgcccacgtgaaggctgccgaccccgggggtggaccatcctctagactggccaccatgcagatcccacaggcgccctggccagtcgtctgggcggtgctacaactgggctggcggccaggatggttcttagactccccagacaggccctggaacccccccaccttctccccagccctgctcgtggtgaccgaaggggacaacgccaccttcacctgcagcttctccaacacatcggagagcttcgtgctaaactggtaccgcatgagccccagcaaccagacggacaagctggccgctttccccgaggaccgcagccagcccggccaggactgccgcttccgtgtcacacaactgcccaacgggcgtgacttccacatgagcgtggtcagggcccggcgcaatgacagcggcacctacctctgtggggccatctccctggcccccaaggcgcagatcaaagagagcctgcgggcagagctcagggtgacagagagaagggcagaagtgcccacagcccaccccagcccctcacccaggccagccggccaggcggccgcacccaccacgacgccagcgccgcgaccaccaaccccggcgcccacgatcgcgtcgcagcccctgtccctgcgcccagaggcgtgccggccagcggcggggggcgcagtgcacacgagggggctggacttcgcctgtgatatctacatctgggcgcccctggccgggacttgtggggtccttctcctgtcactggttatcaccctttactgcaaccacaggcggatccaaggatctggagcaacaaacttctcactactcaaacaagcaggtgacgtggaggagaatcccggccccatggtgagcaagggcgaggaggataacatggccatcatcaaggagttcatgcgcttcaaggtgcacatggagggctccgtgaacggccacgagttcgagatcgagggcgagggcgagggccgcccctacgagggcacccagaccgccaagctgaaggtgaccaagggtggccccctgcccttcgcctgggacatcctgtcccctcagttcatgtacggctccaaggcctacgtgaagcaccccgccgacatccccgactacttgaagctgtccttccccgagggcttcaagtgggagcgcgtgatgaacttcgaggacggcggcgtggtgaccgtgacccaggactcctccctgcaggacggcgagttcatctacaaggtgaagctgcgcggcaccaacttcccctccgacggccccgtaatgcagaagaagaccatgggctgggaggcctcctccgagcggatgtaccccgaggacggcgccctgaagggcgagatcaagcagaggctgaagctgaaggacggcggccactacgacgctgaggtcaagaccacctacaaggccaagaagcccgtgcagctgcccggcgcctacaacgtcaacatcaagttggacatcacctcccacaacgaggactacaccatcgtggaacagtacgaacgcgccgagggccgccactccaccggcggcatggacgagctgtacaagtaactcgag

SEQ ID NO: 48 - protein, 5 aa, Artificial Sequence
  Description of Artificial Sequence: Synthetic peptide
SGGGS